European Patent Application EP 4 413 997 A1, published August 14, 2024. Title: 抗HLA-DQ2.5抗体の製剤. Applicant: CHUGAI SEIYAKU KABUSHIKI KAISHA. Application JP. The sequence listing filed with the application follows.

SEQUENCE LISTING (210 sequences)

SEQ ID NO: 1 - protein, 30 aa, synthetic construct
  REGION 1..30: note = VH1a
QVQLVQSGAEVKKPGSSVKVSCKASGGTFS

SEQ ID NO: 2 - protein, 30 aa, synthetic construct
  REGION 1..30: note = VH1b
QVQLVQSGAEVKKPGASVKVSCKASGYTFT

SEQ ID NO: 3 - protein, 30 aa, synthetic construct
  REGION 1..30: note = VH2
QVQLKESGPALVKPTQTLTLTCTFSGFSLS

SEQ ID NO: 4 - protein, 30 aa, synthetic construct
  REGION 1..30: note = VH3
EVQLVESGGGLVQPGGSLRLSCAASGFTFS

SEQ ID NO: 5 - protein, 30 aa, synthetic construct
  REGION 1..30: note = VH4
QVQLQESGPGLVKPSETLSLTCTVSGGSIS

SEQ ID NO: 6 - protein, 30 aa, synthetic construct
  REGION 1..30: note = VH5
EVQLVQSGAEVKKPGESLKISCKGSGYSFT

SEQ ID NO: 7 - protein, 30 aa, synthetic construct
  REGION 1..30: note = VH6
QVQLQQSGPGLVKPSQTLSLTCAISGDSVS

SEQ ID NO: 8 - skipped

SEQ ID NO: 9 - protein, 14 aa, synthetic construct
  REGION 1..14: note = VH1a
WVRQAPGQGLEWMG

SEQ ID NO: 10 - protein, 14 aa, synthetic construct
  REGION 1..14: note = VH3
WVRQAPGKGLEWVS

SEQ ID NO: 11 - protein, 32 aa, synthetic construct
  REGION 1..32: note = VH1a
RVTITADESTSTAYMELSSLRSEDTAVYYCAR

SEQ ID NO: 12 - protein, 32 aa, synthetic construct
  REGION 1..32: note = VH1b
RVTMTRDTSISTAYMELSSLRSEDTAVYYCAR

SEQ ID NO: 13 - protein, 32 aa, synthetic construct
  REGION 1..32: note = VH2
RLTISKDTSKNQVVLTMTNMDPVDTATYYCAR

SEQ ID NO: 14 - protein, 32 aa, synthetic construct
  REGION 1..32: note = VH3
RFTISRDNSKNTLYLQMNSLRAEDTAVYYCAR

SEQ ID NO: 15 - protein, 32 aa, synthetic construct
  REGION 1..32: note = VH4
RVTISVDTSKNQFSLKLSSVTAADTAVYYCAR

SEQ ID NO: 16 - protein, 32 aa, synthetic construct
  REGION 1..32: note = VH5
QVTISADKSISTAYLQWSSLKASDTAMYYCAR

SEQ ID NO: 17 - protein, 32 aa, synthetic construct
  REGION 1..32: note = VH6
RITINPDTSKNQFSLQLNSVTPEDTAVYYCAR

SEQ ID NO: 18 - protein, 11 aa, synthetic construct
  REGION 1..11: note = VH1a
WGQGTLVTVSS

SEQ ID NO: 19 - protein, 11 aa, synthetic construct
  REGION 1..11: note = VH6
WGPGTLVTVSS

SEQ ID NO: 20 - protein, 23 aa, synthetic construct
  REGION 1..23: note = VK1
DIQMTQSPSSLSASVGDRVTITC

SEQ ID NO: 21 - protein, 23 aa, synthetic construct
  REGION 1..23: note = VK2
DIVMTQSPLSLPVTPGEPASISC

SEQ ID NO: 22 - protein, 23 aa, synthetic construct
  REGION 1..23: note = VK3
DIVLTQSPATLSLSPGERATLSC

SEQ ID NO: 23 - protein, 23 aa, synthetic construct
  REGION 1..23: note = VK4
DIVMTQSPDSLAVSLGERATINC

SEQ ID NO: 24 - protein, 15 aa, synthetic construct
  REGION 1..15: note = VK1
WYQQKPGKAPKLLIY

SEQ ID NO: 25 - skipped

SEQ ID NO: 26 - protein, 32 aa, synthetic construct
  REGION 1..32: note = VK1
GVPSRFSGSGSGTDFTLTISSLQPEDFATYYC

SEQ ID NO: 27 - protein, 32 aa, synthetic construct
  REGION 1..32: note = VK2
GVPDRFSGSGSGTDFTLKISRVEAEDVGVYYC

SEQ ID NO: 28 - protein, 32 aa, synthetic construct
  REGION 1..32: note = VK3
GVPARFSGSGSGTDFTLTISSLEPEDFAVYYC

SEQ ID NO: 29 - protein, 32 aa, synthetic construct
  REGION 1..32: note = VK4
GVPDRFSGSGSGTDFTLTISSLQAEDVAVYYC

SEQ ID NO: 30 - protein, 10 aa, synthetic construct
  REGION 1..10: note = VK1
FGGGTKVEIK

SEQ ID NO: 31 - protein, 328 aa, synthetic construct
  REGION 1..328: note = SG1
ASTKGPSVFPLAPSSKSTSGGTAALGCLVKDYFPEPVTVSWNSGALTSGVHTFPAVLQSSGLYSLSSVVTVPSSSLGTQTYICNVNHKPSNTKVDKKVEPKSCDKTHTCPPCPAPELLGGPSVFLFPPKPKDTLMISRTPEVTCVVVDVSHEDPEVKFNWYVDGVEVHNAKTKPREEQYNSTYRVVSVLTVLHQDWLNGKEYKCKVSNKALPAPIEKTISKAKGQPREPQVYTLPPSREEMTKNQVSLTCLVKGFYPSDIAVEWESNGQPENNYKTTPPVLDSDGSFFLYSKLTVDKSRWQQGNVFSCSVMHEALHNHYTQKSLSLSP

SEQ ID NO: 32 - protein, 107 aa, synthetic construct [sequence omitted]

SEQ ID NO: 33 - protein, 14 aa, synthetic construct
  REGION 1..14: note = VH3 (54H)
WVRQAPGKGLEWVA

SEQ ID NO: 34 - protein, 15 aa, synthetic construct
  REGION 1..15: note = VK4 (38509L)
WYQQKPGQPPKLLIY

SEQ ID NO: 35 - protein, 449 aa, synthetic construct
  REGION 1..449: note = DQN0344Hx-SG1310.A5
QSLEESGGGLVKPGGTLTLTCTASGFSFSSSYWMCWVRQAPGKGLEWVACVYGGSDTTYYASWTKGRFTISKGSSTTVALQVTSLTAADTATYFCARDPLNYYYYGELNLWGPGTLVTVSSASTKGPSVFPLAPSSKSTSGGTAALGCLVKDYFPEPVTVSWNSGALTSGVHTFPAVLKSSGLYSLSSVVTVPSSSLGTQTYICNVNHKPSNTKVDKRVEPKSCDKTHTCPPCPAPELRRGPSVFLFPPKPKDTLMISRTPEVTCVVVDVSHEDPEVKFNWYVDGVEVHNAKTKPREEQYNSTYRVVSVLTVLHQDWLNGKEYKCKVSNKALPAPIEKTISKAKGQPREPQVYTLPPSREEMTKNQVSLTCLVKGFYPSDIAVEWESNGQPENNYKTTPPYLDSDGSFFLYSKLTVDKSRWQEGNVFSCSVLHEALHAHYTREELSLSP

SEQ ID NO: 36 - protein, 449 aa, synthetic construct
  REGION 1..449: note = DQN0344Hx-SG1399.A5
QSLEESGGGLVKPGGTLTLTCTASGFSFSSSYWMCWVRQAPGKGLEWVACVYGGSDTTYYASWTKGRFTISKGSSTTVALQVTSLTAADTATYFCARDPLNYYYYGELNLWGPGTLVTVSSASTKGPSVFPLAPSSKSTSGGTAALGCLVKDYFPEPVTVSWNSGALTSGVHTFPAVLKSSGLYSLSSVVTVPSSSLGTQTYICNVNHKPSNTKVDKRVEPKSCDKTHTCPPCPAPELRRGPSVFLFPPKPKDTLMISRTPEVTCVVVDVSHEDPEVKFNWYVDGVEVHNAKTKPREEQYNSTYRVVSVLTVLHQDWLNGKEYKCKVSNKALPAPIEKTISKAKGQPREPQVYTLPPSREEMTKNQVSLTCLVKGFYPSDIAVEWESNGQPENNYKTTPPVLDSDGSFFLYSKLTVDKSRWQEGNVFSCSVLHEALHAHYTREELSLSP

SEQ ID NO: 37 - protein, 215 aa, synthetic construct
  REGION 1..215: note = DQN0344Lx-SK1004
AVVLTQTASPVSAAVGGTVTIRCQATENIYSGLAWYQQKPGQPPKVLIYYVSTLASGVPSRFKGSGSGTEYTLTISGVQCDDAATYYCQTYHDISNVTFGGGTKVEIKRTVAAPSVFIFPPSDEQLKSGTAEVVCLLNNFYPREAKVQWKVDNALQSGNSEESVTEQDSKDSTYSLSSTLTLSKADYEKHKVYACEVTHQGLSSPVTKSFNRGEC

SEQ ID NO: 38 - protein, 451 aa, synthetic construct
  REGION 1..451: note = DQN034425H-SG1310.A5
QVQLVESGGGVVQPGRSLRLSCAASGFTFSSSYWMCWVRQAPGQGLEWMGCVYGGSDTTYYASWTKGRFTISRDNSKNTLYLQMNSLRAEDTAVYYCARDPLNYYYYGELNLWGQGTLVTVSSASTKGPSVFPLAPSSKSTSGGTAALGCLVKDYFPEPVTVSWNSGALTSGVHTFPAVLKSSGLYSLSSVVTVPSSSLGTQTYICNVNHKPSNTKVDKRVEPKSCDKTHTCPPCPAPELRRGPSVFLFPPKPKDTLMISRTPEVTCVVVDVSHEDPEVKFNWYVDGVEVHNAKTKPREEQYNSTYRVVSVLTVLHQDWLNGKEYKCKVSNKALPAPIEKTISKAKGQPREPQVYTLPPSREEMTKNQVSLTCLVKGFYPSDIAVEWESNGQPENNYKTTPPYLDSDGSFFLYSKLTVDKSRWQEGNVFSCSVLHEALHAHYTREELSLSP

SEQ ID NO: 39 - protein, 451 aa, synthetic construct
  REGION 1..451: note = DQN034425H-SG1399.A5
QVQLVESGGGVVQPGRSLRLSCAASGFTFSSSYWMCWVRQAPGQGLEWMGCVYGGSDTTYYASWTKGRFTISRDNSKNTLYLQMNSLRAEDTAVYYCARDPLNYYYYGELNLWGQGTLVTVSSASTKGPSVFPLAPSSKSTSGGTAALGCLVKDYFPEPVTVSWNSGALTSGVHTFPAVLKSSGLYSLSSVVTVPSSSLGTQTYICNVNHKPSNTKVDKRVEPKSCDKTHTCPPCPAPELRRGPSVFLFPPKPKDTLMISRTPEVTCVVVDVSHEDPEVKFNWYVDGVEVHNAKTKPREEQYNSTYRVVSVLTVLHQDWLNGKEYKCKVSNKALPAPIEKTISKAKGQPREPQVYTLPPSREEMTKNQVSLTCLVKGFYPSDIAVEWESNGQPENNYKTTPPVLDSDGSFFLYSKLTVDKSRWQEGNVFSCSVLHEALHAHYTREELSLSP

SEQ ID NO: 40 - protein, 215 aa, synthetic construct
  REGION 1..215: note = DQN034409L-SK1004
DIQMTQSPSSLSASVGDRVTITCQATENIYSGLAWYQQKPGKAPKLLIYYVSTLASGIPARFSGSGSGTDFTLTISSLEPEDFAVYYCQTYHDISNVTFGQGTKVEIKRTVAAPSVFIFPPSDEQLKSGTAEVVCLLNNFYPREAKVQWKVDNALQSGNSEESVTEQDSKDSTYSLSSTLTLSKADYEKHKVYACEVTHQGLSSPVTKSFNRGEC

SEQ ID NO: 41 - protein, 451 aa, synthetic construct
  REGION 1..451: note = ssVH3.30DQN034425H0976-SG1310.A5
QVQLVESGGGVVQPGGSLRLSCAASGFTFSSAYWMVWVRQAPGQGLEWMGAVYGGSDTTYYAKWTEGRFTISRDTSKNTLYLQMNSLRAEDTAVYYCAREPLNYYYYGELNLWGQGTLVTVSSASTKGPSVFPLAPSSKSTSGGTAALGCLVKDYFPEPVTVSWNSGALTSGVHTFPAVLKSSGLYSLSSVVTVPSSSLGTQTYICNVNHKPSNTKVDKRVEPKSCDKTHTCPPCPAPELRRGPSVFLFPPKPKDTLMISRTPEVTCVVVDVSHEDPEVKFNWYVDGVEVHNAKTKPREEQYNSTYRVVSVLTVLHQDWLNGKEYKCKVSNKALPAPIEKTISKAKGQPREPQVYTLPPSREEMTKNQVSLTCLVKGFYPSDIAVEWESNGQPENNYKTTPPYLDSDGSFFLYSKLTVDKSRWQEGNVFSCSVLHEALHAHYTREELSLSP

SEQ ID NO: 42 - protein, 451 aa, synthetic construct
  REGION 1..451: note = ssVH3.30DQN034425H0976-SG1399.A5
QVQLVESGGGVVQPGGSLRLSCAASGFTFSSAYWMVWVRQAPGQGLEWMGAVYGGSDTTYYAKWTEGRFTISRDTSKNTLYLQMNSLRAEDTAVYYCAREPLNYYYYGELNLWGQGTLVTVSSASTKGPSVFPLAPSSKSTSGGTAALGCLVKDYFPEPVTVSWNSGALTSGVHTFPAVLKSSGLYSLSSVVTVPSSSLGTQTYICNVNHKPSNTKVDKRVEPKSCDKTHTCPPCPAPELRRGPSVFLFPPKPKDTLMISRTPEVTCVVVDVSHEDPEVKFNWYVDGVEVHNAKTKPREEQYNSTYRVVSVLTVLHQDWLNGKEYKCKVSNKALPAPIEKTISKAKGQPREPQVYTLPPSREEMTKNQVSLTCLVKGFYPSDIAVEWESNGQPENNYKTTPPVLDSDGSFFLYSKLTVDKSRWQEGNVFSCSVLHEALHAHYTREELSLSP

SEQ ID NO: 43 - protein, 215 aa, synthetic construct
  REGION 1..215: note = ssVK1.L1DQN034409L0591-SK1004
DIQMTQSPSSLSASVGDRVTITCQATEEIYSGLAWYQQKPGKAPKLLIYYVSTLYEGIPARFSGSGSGTDFTLTISSLEPEDFAVYYCQTYEDVSAVTFGQGTKVEIKRTVAAPSVFIFPPSDEQLKSGTAEVVCLLNNFYPREAKVQWKVDNALQSGNSEESVTEQDSKDSTYSLSSTLTLSKADYEKHKVYACEVTHQGLSSPVTKSFNRGEC

SEQ ID NO: 44 - protein, 451 aa, synthetic construct
  REGION 1..451: note = ssVH3.30DQN034425H1013-SG1310.A5
QVQLVESGGGVVQPGRSLRLSCAASGFTFSSAYWMVWVRQAPGQGLEWMGAVYGGSDTTYYAKWTEGRFTISRDTSKNTLYLQMNSLRAEDTAVYYCAREPLNYYYYGELNVWGQGTLVTVSSASTKGPSVFPLAPSSKSTSGGTAALGCLVKDYFPEPVTVSWNSGALTSGVHTFPAVLKSSGLYSLSSVVTVPSSSLGTQTYICNVNHKPSNTKVDKRVEPKSCDKTHTCPPCPAPELRRGPSVFLFPPKPKDTLMISRTPEVTCVVVDVSHEDPEVKFNWYVDGVEVHNAKTKPREEQYNSTYRVVSVLTVLHQDWLNGKEYKCKVSNKALPAPIEKTISKAKGQPREPQVYTLPPSREEMTKNQVSLTCLVKGFYPSDIAVEWESNGQPENNYKTTPPYLDSDGSFFLYSKLTVDKSRWQEGNVFSCSVLHEALHAHYTREELSLSP

SEQ ID NO: 45 - protein, 451 aa, synthetic construct
  REGION 1..451: note = ssVH3.30DQN034425H1013-SG1399.A5
QVQLVESGGGVVQPGRSLRLSCAASGFTFSSAYWMVWVRQAPGQGLEWMGAVYGGSDTTYYAKWTEGRFTISRDTSKNTLYLQMNSLRAEDTAVYYCAREPLNYYYYGELNVWGQGTLVTVSSASTKGPSVFPLAPSSKSTSGGTAALGCLVKDYFPEPVTVSWNSGALTSGVHTFPAVLKSSGLYSLSSVVTVPSSSLGTQTYICNVNHKPSNTKVDKRVEPKSCDKTHTCPPCPAPELRRGPSVFLFPPKPKDTLMISRTPEVTCVVVDVSHEDPEVKFNWYVDGVEVHNAKTKPREEQYNSTYRVVSVLTVLHQDWLNGKEYKCKVSNKALPAPIEKTISKAKGQPREPQVYTLPPSREEMTKNQVSLTCLVKGFYPSDIAVEWESNGQPENNYKTTPPVLDSDGSFFLYSKLTVDKSRWQEGNVFSCSVLHEALHAHYTREELSLSP

SEQ ID NO: 46 - protein, 215 aa, synthetic construct
  REGION 1..215: note = ssVK1.L1DQN034409L0620-SK1004
DIQMTQSPSSLSASVGDRVTITCQATENIYSGLAWYQQKPGKAPKLLIYYVSTLAYGIPARFSGSGSGTDFTLTISSLEPEDFAVYYCQTYEDVSAVTFGQGTKVEIKRTVAAPSVFIFPPSDEQLKSGTAEVVCLLNNFYPREAKVQWKVDNALQSGNSEESVTEQDSKDSTYSLSSTLTLSKADYEKHKVYACEVTHQGLSSPVTKSFNRGEC

SEQ ID NO: 47 - protein, 445 aa, synthetic construct
  REGION 1..445: note = DQN0385He-SG1308.A5
QEQLEESGGDLVKPGASLTLTCTASGFSFYSSYWICWVRQAPGKGLEWIACIDTGSGSIDYASWVNGRFTISKTSSTTVTLQMTSLTVADTATYFCARDIGIDYNFWGPGTLVTVSSASTKGPSVFPLAPSSKSTSGGTAALGCLVEDYFPEPVTVSWNSGALTSGVHTFPAVLESSGLYSLSSVVTVPSSSLGTKTYICNVNHKPSNTKVDKRVEPKSCDKTHTCPPCPAPELRRGPSVFLFPPKPKDTLMISRTPEVTCVVVDVSHEDPEVKFNWYVDGVEVHNAKTKPREEQYNSTYRVVSVLTVLHQDWLNGKEYKCKVSNKALPAPIEKTISKAKGQPREPQVYTLPPSRKEMTKNQVSLTCLVKGFYPSDIAVEWESNGQPENNYKTTPPYLDSDGSFFLYSKLTVDKSRWQQGNVFSCSVLHEALHAHYTRKELSLSP

SEQ ID NO: 48 - protein, 445 aa, synthetic construct
  REGION 1..445: note = DQN0385He-SG1398.A5
QEQLEESGGDLVKPGASLTLTCTASGFSFYSSYWICWVRQAPGKGLEWIACIDTGSGSIDYASWVNGRFTISKTSSTTVTLQMTSLTVADTATYFCARDIGIDYNFWGPGTLVTVSSASTKGPSVFPLAPSSKSTSGGTAALGCLVEDYFPEPVTVSWNSGALTSGVHTFPAVLESSGLYSLSSVVTVPSSSLGTKTYICNVNHKPSNTKVDKRVEPKSCDKTHTCPPCPAPELRRGPSVFLFPPKPKDTLMISRTPEVTCVVVDVSHEDPEVKFNWYVDGVEVHNAKTKPREEQYNSTYRVVSVLTVLHQDWLNGKEYKCKVSNKALPAPIEKTISKAKGQPREPQVYTLPPSRKEMTKNQVSLTCLVKGFYPSDIAVEWESNGQPENNYKTTPPVLDSDGSFFLYSKLTVDKSRWQQGNVFSCSVLHEALHAHYTRKELSLSP

SEQ ID NO: 49 - protein, 213 aa, synthetic construct
  REGION 1..213: note = DQN0385Le-SK1014
AFELTQTPSFVEAAVGGTVTIKCQATQSISSYLNWYQQKPGQPPKLLIYYASTLASGVPSRFKGSGSGTEFSLTISGVECADAATYYCHYGISYVSFGGGTKVEIKRTVAAPSVFIFPPSDEQLKSGTAKVVCLLNNFYPREAKVQWKVDNALQSGNSKESVTEQDSKDSTYSLSSTLTLSKADYEKHKVYACEVTHQGLSSPVTKSFNRGEC

SEQ ID NO: 50 - protein, 446 aa, synthetic construct
  REGION 1..446: note = DQN0385ee0054H-SG1308.A5
QVQLVESGGGVVQPGRSLRLSCAASGFTFSSSYWICWVRQAPGKGLEWVACIDTGSGSIDYASWVNGRFTISRDNSKNTLYLQMNSLRAEDTAVYYCARDIGIDYNFWGPGTLVTVSSASTKGPSVFPLAPSSKSTSGGTAALGCLVEDYFPEPVTVSWNSGALTSGVHTFPAVLESSGLYSLSSVVTVPSSSLGTKTYICNVNHKPSNTKVDKRVEPKSCDKTHTCPPCPAPELRRGPSVFLFPPKPKDTLMISRTPEVTCVVVDVSHEDPEVKFNWYVDGVEVHNAKTKPREEQYNSTYRVVSVLTVLHQDWLNGKEYKCKVSNKALPAPIEKTISKAKGQPREPQVYTLPPSRKEMTKNQVSLTCLVKGFYPSDIAVEWESNGQPENNYKTTPPYLDSDGSFFLYSKLTVDKSRWQQGNVFSCSVLHEALHAHYTRKELSLSP

SEQ ID NO: 51 - protein, 446 aa, synthetic construct
  REGION 1..446: note = DQN0385ee0054H-SG1398.A5
QVQLVESGGGVVQPGRSLRLSCAASGFTFSSSYWICWVRQAPGKGLEWVACIDTGSGSIDYASWVNGRFTISRDNSKNTLYLQMNSLRAEDTAVYYCARDIGIDYNFWGPGTLVTVSSASTKGPSVFPLAPSSKSTSGGTAALGCLVEDYFPEPVTVSWNSGALTSGVHTFPAVLESSGLYSLSSVVTVPSSSLGTKTYICNVNHKPSNTKVDKRVEPKSCDKTHTCPPCPAPELRRGPSVFLFPPKPKDTLMISRTPEVTCVVVDVSHEDPEVKFNWYVDGVEVHNAKTKPREEQYNSTYRVVSVLTVLHQDWLNGKEYKCKVSNKALPAPIEKTISKAKGQPREPQVYTLPPSRKEMTKNQVSLTCLVKGFYPSDIAVEWESNGQPENNYKTTPPVLDSDGSFFLYSKLTVDKSRWQQGNVFSCSVLHEALHAHYTRKELSLSP

SEQ ID NO: 52 - protein, 213 aa, synthetic construct
  REGION 1..213: note = DQN0385ee009L-SK1014
DIQMTQSPSSLSASVGDRVTITCQATQSISSYLNWYQQKPGQPPKLLIYYASTLASGIPARFSGSGSGTDFTLTISSLEPEDFAVYYCHYGISYVSFGQGTKVEIKRTVAAPSVFIFPPSDEQLKSGTAKVVCLLNNFYPREAKVQWKVDNALQSGNSKESVTEQDSKDSTYSLSSTLTLSKADYEKHKVYACEVTHQGLSSPVTKSFNRGEC

SEQ ID NO: 53 - protein, 446 aa, synthetic construct
  REGION 1..446: note = ssVH3.30DQN0385ee0054H1270-SG1308.A5
QVQLVESGGGVVQPGRSLRLSCAASGFTFSEWYFMSWVRQAPGKGLEWVASIDTGSGSIDYAEWVEGRFTISRDNSKNTLYLQMNSLRAEDTAVYYCARDIGIDYNFWGPGTLVTVSSASTKGPSVFPLAPSSKSTSGGTAALGCLVEDYFPEPVTVSWNSGALTSGVHTFPAVLESSGLYSLSSVVTVPSSSLGTKTYICNVNHKPSNTKVDKRVEPKSCDKTHTCPPCPAPELRRGPSVFLFPPKPKDTLMISRTPEVTCVVVDVSHEDPEVKFNWYVDGVEVHNAKTKPREEQYNSTYRVVSVLTVLHQDWLNGKEYKCKVSNKALPAPIEKTISKAKGQPREPQVYTLPPSRKEMTKNQVSLTCLVKGFYPSDIAVEWESNGQPENNYKTTPPYLDSDGSFFLYSKLTVDKSRWQQGNVFSCSVLHEALHAHYTRKELSLSP

SEQ ID NO: 54 - protein, 446 aa, synthetic construct
  REGION 1..446: note = ssVH3.30DQN0385ee0054H1270-SG1398.A5
QVQLVESGGGVVQPGRSLRLSCAASGFTFSEWYFMSWVRQAPGKGLEWVASIDTGSGSIDYAEWVEGRFTISRDNSKNTLYLQMNSLRAEDTAVYYCARDIGIDYNFWGPGTLVTVSSASTKGPSVFPLAPSSKSTSGGTAALGCLVEDYFPEPVTVSWNSGALTSGVHTFPAVLESSGLYSLSSVVTVPSSSLGTKTYICNVNHKPSNTKVDKRVEPKSCDKTHTCPPCPAPELRRGPSVFLFPPKPKDTLMISRTPEVTCVVVDVSHEDPEVKFNWYVDGVEVHNAKTKPREEQYNSTYRVVSVLTVLHQDWLNGKEYKCKVSNKALPAPIEKTISKAKGQPREPQVYTLPPSRKEMTKNQVSLTCLVKGFYPSDIAVEWESNGQPENNYKTTPPVLDSDGSFFLYSKLTVDKSRWQQGNVFSCSVLHEALHAHYTRKELSLSP

SEQ ID NO: 55 - protein, 213 aa, synthetic construct
  REGION 1..213: note = ssVK1.L1DQN0385ee009L0722-SK1014
DIQMTQSPSSLSASVGDRVTITCQTTQSISSYLNWYQQKPGQPPKLLIYYASTKAEGIPARFSGSGLGTDFTLTISSLQPEDFAVYYCHYGISKVSFGQGTKVEIKRTVAAPSVFIFPPSDEQLKSGTAKVVCLLNNFYPREAKVQWKVDNALQSGNSKESVTEQDSKDSTYSLSSTLTLSKADYEKHKVYACEVTHQGLSSPVTKSFNRGEC

SEQ ID NO: 56 - protein, 213 aa, synthetic construct
  REGION 1..213: note = ssVK1.L1DQN0385ee009L0681-SK1014
DIQMTQSPSSLSASVGDRVTITCQTTQSISSYLNWYQQKPGQPPKLLIYYASTKAEGIPARFSGSGLGTDFTLTISSLEPEDFAVYYCHYGISKVSFGQGTKVEIKRTVAAPSVFIFPPSDEQLKSGTAKVVCLLNNFYPREAKVQWKVDNALQSGNSKESVTEQDSKDSTYSLSSTLTLSKADYEKHKVYACEVTHQGLSSPVTKSFNRGEC

SEQ ID NO: 57 - protein, 446 aa, synthetic construct
  REGION 1..446: note = ssVH3.30DQN0385ee0054H1352-SG1308.A5
QVQLVESGGGVVQPGRSLRLSCAASGFEFSEWYFMSWVRQAPGKGLEWVASIDTGSGSIDYAEWVEGRFTISRDNSKNTLYLQMNSLRAEDTAVYYCARDIGIDYNFWGPGTLVTVSSASTKGPSVFPLAPSSKSTSGGTAALGCLVEDYFPEPVTVSWNSGALTSGVHTFPAVLESSGLYSLSSVVTVPSSSLGTKTYICNVNHKPSNTKVDKRVEPKSCDKTHTCPPCPAPELRRGPSVFLFPPKPKDTLMISRTPEVTCVVVDVSHEDPEVKFNWYVDGVEVHNAKTKPREEQYNSTYRVVSVLTVLHQDWLNGKEYKCKVSNKALPAPIEKTISKAKGQPREPQVYTLPPSRKEMTKNQVSLTCLVKGFYPSDIAVEWESNGQPENNYKTTPPYLDSDGSFFLYSKLTVDKSRWQQGNVFSCSVLHEALHAHYTRKELSLSP

SEQ ID NO: 58 - protein, 446 aa, synthetic construct
  REGION 1..446: note = ssVH3.30DQN0385ee0054H1352-SG1398.A5
QVQLVESGGGVVQPGRSLRLSCAASGFEFSEWYFMSWVRQAPGKGLEWVASIDTGSGSIDYAEWVEGRFTISRDNSKNTLYLQMNSLRAEDTAVYYCARDIGIDYNFWGPGTLVTVSSASTKGPSVFPLAPSSKSTSGGTAALGCLVEDYFPEPVTVSWNSGALTSGVHTFPAVLESSGLYSLSSVVTVPSSSLGTKTYICNVNHKPSNTKVDKRVEPKSCDKTHTCPPCPAPELRRGPSVFLFPPKPKDTLMISRTPEVTCVVVDVSHEDPEVKFNWYVDGVEVHNAKTKPREEQYNSTYRVVSVLTVLHQDWLNGKEYKCKVSNKALPAPIEKTISKAKGQPREPQVYTLPPSRKEMTKNQVSLTCLVKGFYPSDIAVEWESNGQPENNYKTTPPVLDSDGSFFLYSKLTVDKSRWQQGNVFSCSVLHEALHAHYTRKELSLSP

SEQ ID NO: 59 - protein, 446 aa, synthetic construct
  REGION 1..446: note = ssVH3.30DQN0385ee0054H1527-SG1308.A5
QVQLVESGGGVVQPGRSLRLSCAASGFTFASWYFMSWVRQAPGKGLEWVASIDTGSGSIDYAEWVEGRFTISRDNSKNTLYLQMNSLRAEDTAVYYCARDIGIDYNFWGPGTLVTVSSASTKGPSVFPLAPSSKSTSGGTAALGCLVEDYFPEPVTVSWNSGALTSGVHTFPAVLESSGLYSLSSVVTVPSSSLGTKTYICNVNHKPSNTKVDKRVEPKSCDKTHTCPPCPAPELRRGPSVFLFPPKPKDTLMISRTPEVTCVVVDVSHEDPEVKFNWYVDGVEVHNAKTKPREEQYNSTYRVVSVLTVLHQDWLNGKEYKCKVSNKALPAPIEKTISKAKGQPREPQVYTLPPSRKEMTKNQVSLTCLVKGFYPSDIAVEWESNGQPENNYKTTPPYLDSDGSFFLYSKLTVDKSRWQQGNVFSCSVLHEALHAHYTRKELSLSP

SEQ ID NO: 60 - protein, 446 aa, synthetic construct
  REGION 1..446: note = ssVH3.30DQN0385ee0054H1527-SG1398.A5
QVQLVESGGGVVQPGRSLRLSCAASGFTFASWYFMSWVRQAPGKGLEWVASIDTGSGSIDYAEWVEGRFTISRDNSKNTLYLQMNSLRAEDTAVYYCARDIGIDYNFWGPGTLVTVSSASTKGPSVFPLAPSSKSTSGGTAALGCLVEDYFPEPVTVSWNSGALTSGVHTFPAVLESSGLYSLSSVVTVPSSSLGTKTYICNVNHKPSNTKVDKRVEPKSCDKTHTCPPCPAPELRRGPSVFLFPPKPKDTLMISRTPEVTCVVVDVSHEDPEVKFNWYVDGVEVHNAKTKPREEQYNSTYRVVSVLTVLHQDWLNGKEYKCKVSNKALPAPIEKTISKAKGQPREPQVYTLPPSRKEMTKNQVSLTCLVKGFYPSDIAVEWESNGQPENNYKTTPPVLDSDGSFFLYSKLTVDKSRWQQGNVFSCSVLHEALHAHYTRKELSLSP

SEQ ID NO: 61 - protein, 213 aa, synthetic construct
  REGION 1..213: note = ssVK1.L1DQN0385ee009L0605-SK1014
DIQMTQSPSSLSASVGDRVTITCQTTQSISSYLNWYQQKPGQPPKLLIYYASTKAEGIPARFSGSGSGTDFTLTISSLEPEDFAVYYCHYGISKVSFGQGTKVEIKRTVAAPSVFIFPPSDEQLKSGTAKVVCLLNNFYPREAKVQWKVDNALQSGNSKESVTEQDSKDSTYSLSSTLTLSKADYEKHKVYACEVTHQGLSSPVTKSFNRGEC

SEQ ID NO: 62 - protein, 446 aa, synthetic construct
  REGION 1..446: note = ssVH3.30DQN0385ee0054H1255-SG1308.A5
QVQLVESGGGVVQPGRSLRLSCAASGFTFSEWYFMSWVRQAPGKGLEWVASIDTGSGSIDYAGWVEERFTISRDNSKNTLYLQMNSLRAEDTAVYYCARDIGIDYNFWGPGTLVTVSSASTKGPSVFPLAPSSKSTSGGTAALGCLVEDYFPEPVTVSWNSGALTSGVHTFPAVLESSGLYSLSSVVTVPSSSLGTKTYICNVNHKPSNTKVDKRVEPKSCDKTHTCPPCPAPELRRGPSVFLFPPKPKDTLMISRTPEVTCVVVDVSHEDPEVKFNWYVDGVEVHNAKTKPREEQYNSTYRVVSVLTVLHQDWLNGKEYKCKVSNKALPAPIEKTISKAKGQPREPQVYTLPPSRKEMTKNQVSLTCLVKGFYPSDIAVEWESNGQPENNYKTTPPYLDSDGSFFLYSKLTVDKSRWQQGNVFSCSVLHEALHAHYTRKELSLSP

SEQ ID NO: 63 - protein, 446 aa, synthetic construct
  REGION 1..446: note = ssVH3.30DQN0385ee0054H1255-SG1398.A5
QVQLVESGGGVVQPGRSLRLSCAASGFTFSEWYFMSWVRQAPGKGLEWVASIDTGSGSIDYAGWVEERFTISRDNSKNTLYLQMNSLRAEDTAVYYCARDIGIDYNFWGPGTLVTVSSASTKGPSVFPLAPSSKSTSGGTAALGCLVEDYFPEPVTVSWNSGALTSGVHTFPAVLESSGLYSLSSVVTVPSSSLGTKTYICNVNHKPSNTKVDKRVEPKSCDKTHTCPPCPAPELRRGPSVFLFPPKPKDTLMISRTPEVTCVVVDVSHEDPEVKFNWYVDGVEVHNAKTKPREEQYNSTYRVVSVLTVLHQDWLNGKEYKCKVSNKALPAPIEKTISKAKGQPREPQVYTLPPSRKEMTKNQVSLTCLVKGFYPSDIAVEWESNGQPENNYKTTPPVLDSDGSFFLYSKLTVDKSRWQQGNVFSCSVLHEALHAHYTRKELSLSP

SEQ ID NO: 64 - protein, 446 aa, synthetic construct
  REGION 1..446: note = sVH3.30DQN0385ee0054H1521-SG1308.A5
QVQLVESGGGVVQPGRSLRLSCAASGFTFESWYFMSWVRQAPGKGLEWVASIDTGSGSIDYAEWVEGRFTISRDNSKNTLYLQMNSLRAEDTAVYYCARDIGIDYNFWGPGTLVTVSSASTKGPSVFPLAPSSKSTSGGTAALGCLVEDYFPEPVTVSWNSGALTSGVHTFPAVLESSGLYSLSSVVTVPSSSLGTKTYICNVNHKPSNTKVDKRVEPKSCDKTHTCPPCPAPELRRGPSVFLFPPKPKDTLMISRTPEVTCVVVDVSHEDPEVKFNWYVDGVEVHNAKTKPREEQYNSTYRVVSVLTVLHQDWLNGKEYKCKVSNKALPAPIEKTISKAKGQPREPQVYTLPPSRKEMTKNQVSLTCLVKGFYPSDIAVEWESNGQPENNYKTTPPYLDSDGSFFLYSKLTVDKSRWQQGNVFSCSVLHEALHAHYTRKELSLSP

SEQ ID NO: 65 - protein, 446 aa, synthetic construct
  REGION 1..446: note = ssVH3.30DQN0385ee0054H1521-SG1398.A5
QVQLVESGGGVVQPGRSLRLSCAASGFTFESWYFMSWVRQAPGKGLEWVASIDTGSGSIDYAEWVEGRFTISRDNSKNTLYLQMNSLRAEDTAVYYCARDIGIDYNFWGPGTLVTVSSASTKGPSVFPLAPSSKSTSGGTAALGCLVEDYFPEPVTVSWNSGALTSGVHTFPAVLESSGLYSLSSVVTVPSSSLGTKTYICNVNHKPSNTKVDKRVEPKSCDKTHTCPPCPAPELRRGPSVFLFPPKPKDTLMISRTPEVTCVVVDVSHEDPEVKFNWYVDGVEVHNAKTKPREEQYNSTYRVVSVLTVLHQDWLNGKEYKCKVSNKALPAPIEKTISKAKGQPREPQVYTLPPSRKEMTKNQVSLTCLVKGFYPSDIAVEWESNGQPENNYKTTPPVLDSDGSFFLYSKLTVDKSRWQQGNVFSCSVLHEALHAHYTRKELSLSP

SEQ ID NO: 66 - protein, 446 aa, synthetic construct
  REGION 1..446: note = ssVH3.30DQN0385ee0054H1353-SG1308.A5
QVQLVESGGGVVQPGRSLRLSCAASGFTFAEWYFMSWVRQAPGKGLEWVASIDTGSGSIDYAEWVEGRFTISRDNSKNTLYLQMNSLRAEDTAVYYCARDIGIDYNFWGPGTLVTVSSASTKGPSVFPLAPSSKSTSGGTAALGCLVEDYFPEPVTVSWNSGALTSGVHTFPAVLESSGLYSLSSVVTVPSSSLGTKTYICNVNHKPSNTKVDKRVEPKSCDKTHTCPPCPAPELRRGPSVFLFPPKPKDTLMISRTPEVTCVVVDVSHEDPEVKFNWYVDGVEVHNAKTKPREEQYNSTYRVVSVLTVLHQDWLNGKEYKCKVSNKALPAPIEKTISKAKGQPREPQVYTLPPSRKEMTKNQVSLTCLVKGFYPSDIAVEWESNGQPENNYKTTPPYLDSDGSFFLYSKLTVDKSRWQQGNVFSCSVLHEALHAHYTRKELSLSP

SEQ ID NO: 67 - protein, 446 aa, synthetic construct
  REGION 1..446: note = ssVH3.30DQN0385ee0054H1353-SG1398.A5
QVQLVESGGGVVQPGRSLRLSCAASGFTFAEWYFMSWVRQAPGKGLEWVASIDTGSGSIDYAEWVEGRFTISRDNSKNTLYLQMNSLRAEDTAVYYCARDIGIDYNFWGPGTLVTVSSASTKGPSVFPLAPSSKSTSGGTAALGCLVEDYFPEPVTVSWNSGALTSGVHTFPAVLESSGLYSLSSVVTVPSSSLGTKTYICNVNHKPSNTKVDKRVEPKSCDKTHTCPPCPAPELRRGPSVFLFPPKPKDTLMISRTPEVTCVVVDVSHEDPEVKFNWYVDGVEVHNAKTKPREEQYNSTYRVVSVLTVLHQDWLNGKEYKCKVSNKALPAPIEKTISKAKGQPREPQVYTLPPSRKEMTKNQVSLTCLVKGFYPSDIAVEWESNGQPENNYKTTPPVLDSDGSFFLYSKLTVDKSRWQQGNVFSCSVLHEALHAHYTRKELSLSP

SEQ ID NO: 68 - protein, 6 aa, synthetic construct
  REGION 1..6: note = DQN0344Hx H_CDR1
SSYWMC

SEQ ID NO: 69 - protein, 17 aa, synthetic construct
  REGION 1..17: note = DQN0344Hx H_CDR2
CVYGGSDTTYYASWTKG

SEQ ID NO: 70 - protein, 13 aa, synthetic construct
  REGION 1..13: note = DQN0344Hx H_CDR3
DPLNYYYYGELNL

SEQ ID NO: 71 - protein, 121 aa, synthetic construct
  REGION 1..121: note = DQN0344Hx
QSLEESGGGLVKPGGTLTLTCTASGFSFSSSYWMCWVRQAPGKGLEWVACVYGGSDTTYYASWTKGRFTISKGSSTTVALQVTSLTAADTATYFCARDPLNYYYYGELNLWGPGTLVTVSS

SEQ ID NO: 72 - protein, 11 aa, synthetic construct
  REGION 1..11: note = DQN0344Lx L_CDR1
QATENIYSGLA

SEQ ID NO: 73 - protein, 7 aa, synthetic construct
  REGION 1..7: note = DQN0344Lx L_CDR2
YVSTLAS

SEQ ID NO: 74 - protein, 10 aa, synthetic construct
  REGION 1..10: note = DQN0344Lx L_CDR3
QTYHDISNVT

SEQ ID NO: 75 - protein, 108 aa, synthetic construct
  REGION 1..108: note = DQN0344Lx
AVVLTQTASPVSAAVGGTVTIRCQATENIYSGLAWYQQKPGQPPKVLIYYVSTLASGVPSRFKGSGSGTEYTLTISGVQCDDAATYYCQTYHDISNVTFGGGTKVEIK

SEQ ID NO: 76 - protein, 6 aa, synthetic construct
  REGION 1..6: note = DQN0385He H_CDR1
SSYWIC

SEQ ID NO: 77 - protein, 17 aa, synthetic construct
  REGION 1..17: note = DQN0385He H_CDR2
CIDTGSGSIDYASWVNG

SEQ ID NO: 78 - protein, 8 aa, synthetic construct
  REGION 1..8: note = DQN0385He H_CDR3
DIGIDYNF

SEQ ID NO: 79 - protein, 117 aa, synthetic construct
  REGION 1..117: note = DQN0385He
QEQLEESGGDLVKPGASLTLTCTASGFSFYSSYWICWVRQAPGKGLEWIACIDTGSGSIDYASWVNGRFTISKTSSTTVTLQMTSLTVADTATYFCARDIGIDYNFWGPGTLVTVSS

SEQ ID NO: 80 - protein, 11 aa, synthetic construct
  REGION 1..11: note = DQN0385Le L_CDR1
QATQSISSYLN

SEQ ID NO: 81 - protein, 7 aa, synthetic construct
  REGION 1..7: note = DQN0385Le L_CDR2
YASTLAS

SEQ ID NO: 82 - protein, 8 aa, synthetic construct
  REGION 1..8: note = DQN0385Le L_CDR3
HYGISYVS

SEQ ID NO: 83 - protein, 106 aa, synthetic construct
  REGION 1..106: note = DQN0385Le
AFELTQTPSFVEAAVGGTVTIKCQATQSISSYLNWYQQKPGQPPKLLIYYASTLASGVPSRFKGSGSGTEFSLTISGVECADAATYYCHYGISYVSFGGGTKVEIK

SEQ ID NO: 84 - protein, 123 aa, synthetic construct
  REGION 1..123: note = DQN034425H
QVQLVESGGGVVQPGRSLRLSCAASGFTFSSSYWMCWVRQAPGQGLEWMGCVYGGSDTTYYASWTKGRFTISRDNSKNTLYLQMNSLRAEDTAVYYCARDPLNYYYYGELNLWGQGTLVTVSS

SEQ ID NO: 85 - protein, 108 aa, synthetic construct
  REGION 1..108: note = DQN034409L
DIQMTQSPSSLSASVGDRVTITCQATENIYSGLAWYQQKPGKAPKLLIYYVSTLASGIPARFSGSGSGTDFTLTISSLEPEDFAVYYCQTYHDISNVTFGQGTKVEIK

SEQ ID NO: 86 - protein, 106 aa, synthetic construct
  REGION 1..106: note = DQN0385ee009L
DIQMTQSPSSLSASVGDRVTITCQATQSISSYLNWYQQKPGQPPKLLIYYASTLASGIPARFSGSGSGTDFTLTISSLEPEDFAVYYCHYGISYVSFGQGTKVEIK

SEQ ID NO: 87 - protein, 118 aa, synthetic construct
  REGION 1..118: note = DQN0385ee0054H
QVQLVESGGGVVQPGRSLRLSCAASGFTFSSSYWICWVRQAPGKGLEWVACIDTGSGSIDYASWVNGRFTISRDNSKNTLYLQMNSLRAEDTAVYYCARDIGIDYNFWGPGTLVTVSS

SEQ ID NO: 88 - protein, 123 aa, synthetic construct
  REGION 1..123: note = DQN0344H0976
QVQLVESGGGVVQPGGSLRLSCAASGFTFSSAYWMVWVRQAPGQGLEWMGAVYGGSDTTYYAKWTEGRFTISRDTSKNTLYLQMNSLRAEDTAVYYCAREPLNYYYYGELNLWGQGTLVTVSS

SEQ ID NO: 89 - protein, 123 aa, synthetic construct
  REGION 1..123: note = DQN0344H1013
QVQLVESGGGVVQPGRSLRLSCAASGFTFSSAYWMVWVRQAPGQGLEWMGAVYGGSDTTYYAKWTEGRFTISRDTSKNTLYLQMNSLRAEDTAVYYCAREPLNYYYYGELNVWGQGTLVTVSS

SEQ ID NO: 90 - protein, 108 aa, synthetic construct
  REGION 1..108: note = DQN0344L0591
DIQMTQSPSSLSASVGDRVTITCQATEEIYSGLAWYQQKPGKAPKLLIYYVSTLYEGIPARFSGSGSGTDFTLTISSLEPEDFAVYYCQTYEDVSAVTFGQGTKVEIK

SEQ ID NO: 91 - protein, 108 aa, synthetic construct
  REGION 1..108: note = DQN0344L0620
DIQMTQSPSSLSASVGDRVTITCQATENIYSGLAWYQQKPGKAPKLLIYYVSTLAYGIPARFSGSGSGTDFTLTISSLEPEDFAVYYCQTYEDVSAVTFGQGTKVEIK

SEQ ID NO: 92 - protein, 118 aa, synthetic construct
  REGION 1..118: note = DQN0385H1270
QVQLVESGGGVVQPGRSLRLSCAASGFTFSEWYFMSWVRQAPGKGLEWVASIDTGSGSIDYAEWVEGRFTISRDNSKNTLYLQMNSLRAEDTAVYYCARDIGIDYNFWGPGTLVTVSS

SEQ ID NO: 93 - protein, 118 aa, synthetic construct
  REGION 1..118: note = DQN0385H1352
QVQLVESGGGVVQPGRSLRLSCAASGFEFSEWYFMSWVRQAPGKGLEWVASIDTGSGSIDYAEWVEGRFTISRDNSKNTLYLQMNSLRAEDTAVYYCARDIGIDYNFWGPGTLVTVSS

SEQ ID NO: 94 - protein, 118 aa, synthetic construct
  REGION 1..118: note = DQN0385H1527
QVQLVESGGGVVQPGRSLRLSCAASGFTFASWYFMSWVRQAPGKGLEWVASIDTGSGSIDYAEWVEGRFTISRDNSKNTLYLQMNSLRAEDTAVYYCARDIGIDYNFWGPGTLVTVSS

SEQ ID NO: 95 - protein, 118 aa, synthetic construct
  REGION 1..118: note = DQN0385H1255
QVQLVESGGGVVQPGRSLRLSCAASGFTFSEWYFMSWVRQAPGKGLEWVASIDTGSGSIDYAGWVEERFTISRDNSKNTLYLQMNSLRAEDTAVYYCARDIGIDYNFWGPGTLVTVSS

SEQ ID NO: 96 - protein, 118 aa, synthetic construct
  REGION 1..118: note = DQN0385H1521
QVQLVESGGGVVQPGRSLRLSCAASGFTFESWYFMSWVRQAPGKGLEWVASIDTGSGSIDYAEWVEGRFTISRDNSKNTLYLQMNSLRAEDTAVYYCARDIGIDYNFWGPGTLVTVSS

SEQ ID NO: 97 - protein, 118 aa, synthetic construct
  REGION 1..118: note = DQN0385H1353
QVQLVESGGGVVQPGRSLRLSCAASGFTFAEWYFMSWVRQAPGKGLEWVASIDTGSGSIDYAEWVEGRFTISRDNSKNTLYLQMNSLRAEDTAVYYCARDIGIDYNFWGPGTLVTVSS

SEQ ID NO: 98 - protein, 106 aa, synthetic construct
  REGION 1..106: note = DQN0385L0722
DIQMTQSPSSLSASVGDRVTITCQTTQSISSYLNWYQQKPGQPPKLLIYYASTKAEGIPARFSGSGLGTDFTLTISSLQPEDFAVYYCHYGISKVSFGQGTKVEIK

SEQ ID NO: 99 - protein, 106 aa, synthetic construct
  REGION 1..106: note = DQN0385L0681
DIQMTQSPSSLSASVGDRVTITCQTTQSISSYLNWYQQKPGQPPKLLIYYASTKAEGIPARFSGSGLGTDFTLTISSLEPEDFAVYYCHYGISKVSFGQGTKVEIK

SEQ ID NO: 100 - protein, 106 aa, synthetic construct
  REGION 1..106: note = DQN0385L0605
DIQMTQSPSSLSASVGDRVTITCQTTQSISSYLNWYQQKPGQPPKLLIYYASTKAEGIPARFSGSGSGTDFTLTISSLEPEDFAVYYCHYGISKVSFGQGTKVEIK

SEQ ID NO: 101 - protein, 328 aa, synthetic construct
  REGION 1..328: note = SG181.S3n
ASTKGPSVFPLAPSSKSTSGGTAALGCLVKDYFPEPVTVSWNSGALTSGVHTFPAVLQSSGLYSLSSVVTVPSSSLGTQTYICNVNHKPSNTKVDKRVEPKSCDKTHTCPPCPAPELRRGPSVFLFPPKPKDTLMISRTPEVTCVVVDVSHEDPEVKFNWYVDGVEVHNAKTKPREEQYNSTYRVVSVLTVLHQDWLNGKEYKCKVSNKALPAPIEKTISKAKGQPREPQVYTLPPSREEMTKNQVSLTCLVKGFYPSDIAVEWESNGQPENNYKTTPPYLDSDGSFFLYSKLTVDKSRWQQGNVFSCSVMHEALHNHYTQESLSLSP

SEQ ID NO: 102 - protein, 328 aa, synthetic construct
  REGION 1..328: note = SG181.S3p
ASTKGPSVFPLAPSSKSTSGGTAALGCLVKDYFPEPVTVSWNSGALTSGVHTFPAVLQSSGLYSLSSVVTVPSSSLGTQTYICNVNHKPSNTKVDKRVEPKSCDKTHTCPPCPAPELRRGPSVFLFPPKPKDTLMISRTPEVTCVVVDVSHEDPEVKFNWYVDGVEVHNAKTKPREEQYNSTYRVVSVLTVLHQDWLNGKEYKCKVSNKALPAPIEKTISKAKGQPREPQVYTLPPSRKEMTKNQVSLTCLVKGFYPSDIAVEWESNGQPENNYKTTPPYLDSDGSFFLYSKLTVDKSRWQQGNVFSCSVMHEALHNHYTQKSLSLSP

SEQ ID NO: 103 - protein, 107 aa, synthetic construct [sequence omitted]

SEQ ID NO: 104 - protein, 328 aa, synthetic construct
  REGION 1..328: note = SG1308.A5
ASTKGPSVFPLAPSSKSTSGGTAALGCLVEDYFPEPVTVSWNSGALTSGVHTFPAVLESSGLYSLSSVVTVPSSSLGTKTYICNVNHKPSNTKVDKRVEPKSCDKTHTCPPCPAPELRRGPSVFLFPPKPKDTLMISRTPEVTCVVVDVSHEDPEVKFNWYVDGVEVHNAKTKPREEQYNSTYRVVSVLTVLHQDWLNGKEYKCKVSNKALPAPIEKTISKAKGQPREPQVYTLPPSRKEMTKNQVSLTCLVKGFYPSDIAVEWESNGQPENNYKTTPPYLDSDGSFFLYSKLTVDKSRWQQGNVFSCSVLHEALHAHYTRKELSLSP

SEQ ID NO: 105 - protein, 328 aa, synthetic construct
  REGION 1..328: note = SG1310.A5
ASTKGPSVFPLAPSSKSTSGGTAALGCLVKDYFPEPVTVSWNSGALTSGVHTFPAVLKSSGLYSLSSVVTVPSSSLGTQTYICNVNHKPSNTKVDKRVEPKSCDKTHTCPPCPAPELRRGPSVFLFPPKPKDTLMISRTPEVTCVVVDVSHEDPEVKFNWYVDGVEVHNAKTKPREEQYNSTYRVVSVLTVLHQDWLNGKEYKCKVSNKALPAPIEKTISKAKGQPREPQVYTLPPSREEMTKNQVSLTCLVKGFYPSDIAVEWESNGQPENNYKTTPPYLDSDGSFFLYSKLTVDKSRWQEGNVFSCSVLHEALHAHYTREELSLSP

SEQ ID NO: 106 - protein, 107 aa, synthetic construct
  REGION 1..107: note = SK1004
RTVAAPSVFIFPPSDEQLKSGTAEVVCLLNNFYPREAKVQWKVDNALQSGNSEESVTEQDSKDSTYSLSSTLTLSKADYEKHKVYACEVTHQGLSSPVTKSFNRGEC

SEQ ID NO: 107 - protein, 107 aa, synthetic construct
  REGION 1..107: note = SK1014
RTVAAPSVFIFPPSDEQLKSGTAKVVCLLNNFYPREAKVQWKVDNALQSGNSKESVTEQDSKDSTYSLSSTLTLSKADYEKHKVYACEVTHQGLSSPVTKSFNRGEC

SEQ ID NO: 108 - protein, 11 aa, synthetic construct
  REGION 1..11: note = DQN034409L0012 L_CDR1
QATENIYSGLA

SEQ ID NO: 109 - protein, 7 aa, synthetic construct
  REGION 1..7: note = DQN034409L0012 L_CDR2
YVSTLAS

SEQ ID NO: 110 - protein, 10 aa, synthetic construct
  REGION 1..10: note = DQN034409L0012 L_CDR3
QTYHDISEVT

SEQ ID NO: 111 - protein, 108 aa, synthetic construct
  REGION 1..108: note = DQN034409L0012
DIQMTQSPSSLSASVGDRVTITCQATENIYSGLAWYQQKPGKAPKLLIYYVSTLASGIPARFSGSGSGTDFTLTISSLEPEDFAVYYCQTYHDISEVTFGQGTKVEIK

SEQ ID NO: 112 - protein, 6 aa, synthetic construct
  REGION 1..6: note = DQN034425H H_CDR1
SSYWMC

SEQ ID NO: 113 - protein, 17 aa, synthetic construct
  REGION 1..17: note = DQN034425H H_CDR2
CVYGGSDTTYYASWTKG

SEQ ID NO: 114 - protein, 13 aa, synthetic construct
  REGION 1..13: note = DQN034425H H_CDR3
DPLNYYYYGELNL

SEQ ID NO: 115 - protein, 6 aa, synthetic construct
  REGION 1..6: note = DQN0385ee0054H H_CDR1
SSYWIC

SEQ ID NO: 116 - protein, 17 aa, synthetic construct
  REGION 1..17: note = DQN0385ee0054H H_CDR2
CIDTGSGSIDYASWVNG

SEQ ID NO: 117 - protein, 8 aa, synthetic construct
  REGION 1..8: note = DQN0385ee0054H H_CDR3
DIGIDYNF

SEQ ID NO: 118 - protein, 11 aa, synthetic construct
  REGION 1..11: note = DQN0385ee009L L_CDR1
QATQSISSYLN

SEQ ID NO: 119 - protein, 7 aa, synthetic construct
  REGION 1..7: note = DQN0385ee009L L_CDR2
YASTLAS

SEQ ID NO: 120 - protein, 8 aa, synthetic construct
  REGION 1..8: note = DQN0385ee009L L_CDR3
HYGISYVS

SEQ ID NO: 121 - protein, 5 aa, synthetic construct
  REGION 1..5: note = IC17HdK H_CDR1
SYWMH

SEQ ID NO: 122 - protein, 17 aa, synthetic construct
  REGION 1..17: note = IC17HdK H_CDR2
MIDPSYSETRLNQKFKD

SEQ ID NO: 123 - protein, 7 aa, synthetic construct
  REGION 1..7: note = IC17HdK H_CDR3
YGNYFDY

SEQ ID NO: 124 - protein, 116 aa, synthetic construct
  REGION 1..116: note = IC17HdK
QVQLQQSGPQLVRPGASVKISCKASGYSFTSYWMHWVNQRPGQGLEWIGMIDPSYSETRLNQKFKDKATLTVDKSSSTAYMQLSSPTSEDSAVYYCALYGNYFDYWGQGTTLTVSS

SEQ ID NO: 125 - protein, 11 aa, synthetic construct
  REGION 1..11: note = IC17L L_CDR1
KASEDIYNRLA

SEQ ID NO: 126 - protein, 7 aa, synthetic construct
  REGION 1..7: note = IC17L L_CDR2
GATSLET

SEQ ID NO: 127 - protein, 9 aa, synthetic construct
  REGION 1..9: note = IC17L L_CDR3
QQYWSTPYT

SEQ ID NO: 128 - protein, 107 aa, synthetic construct
  REGION 1..107: note = IC17L
DIQMTQSSSSFSVSLGDRVTITCKASEDIYNRLAWYQQKPGNAPRLLISGATSLETGVPSRFSGSGSGKDYTLSITSLQTEDVATYYCQQYWSTPYTFGGGTKLEVK

SEQ ID NO: 129 - protein, 6 aa, synthetic construct
  REGION 1..6: note = DQN0344H0976 H_CDR1
SAYWMV

SEQ ID NO: 130 - protein, 17 aa, synthetic construct
  REGION 1..17: note = DQN0344H0976 H_CDR2
AVYGGSDTTYYAKWTEG

SEQ ID NO: 131 - protein, 13 aa, synthetic construct
  REGION 1..13: note = DQN0344H0976 H_CDR3
EPLNYYYYGELNL

SEQ ID NO: 132 - protein, 11 aa, synthetic construct
  REGION 1..11: note = DQN0344L0591 L_CDR1
QATEEIYSGLA

SEQ ID NO: 133 - protein, 7 aa, synthetic construct
  REGION 1..7: note = DQN0344L0591 L_CDR2
YVSTLYE

SEQ ID NO: 134 - protein, 10 aa, synthetic construct
  REGION 1..10: note = DQN0344L0591 L_CDR3
QTYEDVSAVT

SEQ ID NO: 135 - protein, 6 aa, synthetic construct
  REGION 1..6: note = DQN0385H1270 H_CDR1
EWYFMS

SEQ ID NO: 136 - protein, 17 aa, synthetic construct
  REGION 1..17: note = DQN0385H1270 H_CDR2
SIDTGSGSIDYAEWVEG

SEQ ID NO: 137 - protein, 8 aa, synthetic construct
  REGION 1..8: note = DQN0385H1270 H_CDR3
DIGIDYNF

SEQ ID NO: 138 - protein, 11 aa, synthetic construct
  REGION 1..11: note = DQN0385L0722 L_CDR1
QTTQSISSYLN

SEQ ID NO: 139 - protein, 7 aa, synthetic construct
  REGION 1..7: note = DQN0385L0722 L_CDR2
YASTKAE

SEQ ID NO: 140 - protein, 8 aa, synthetic construct
  REGION 1..8: note = DQN0385L0722 L_CDR3
HYGISKVS

SEQ ID NO: 141 - protein, 11 aa, synthetic construct
  REGION 1..11: note = DQN0385L0681 L_CDR1
QTTQSISSYLN

SEQ ID NO: 142 - protein, 7 aa, synthetic construct
  REGION 1..7: note = DQN0385L0681 L_CDR2
YASTKAE

SEQ ID NO: 143 - protein, 8 aa, synthetic construct
  REGION 1..8: note = DQN0385L0681 L_CDR3
HYGISKVS

SEQ ID NO: 144 - protein, 6 aa, synthetic construct
  REGION 1..6: note = DQN0385H1352 H_CDR1
EWYFMS

SEQ ID NO: 145 - protein, 17 aa, synthetic construct
  REGION 1..17: note = DQN0385H1352 H_CDR2
SIDTGSGSIDYAEWVEG

SEQ ID NO: 146 - protein, 8 aa, synthetic construct
  REGION 1..8: note = DQN0385H1352 H_CDR3
DIGIDYNF

SEQ ID NO: 147 - protein, 6 aa, synthetic construct
  REGION 1..6: note = DQN0385H1527 H_CDR1
SWYFMS

SEQ ID NO: 148 - protein, 17 aa, synthetic construct
  REGION 1..17: note = DQN0385H1527 H_CDR2
SIDTGSGSIDYAEWVEG

SEQ ID NO: 149 - protein, 8 aa, synthetic construct
  REGION 1..8: note = DQN0385H1527 H_CDR3
DIGIDYNF

SEQ ID NO: 150 - protein, 11 aa, synthetic construct
  REGION 1..11: note = DQN0385L0605 L_CDR1
QTTQSISSYLN

SEQ ID NO: 151 - protein, 7 aa, synthetic construct
  REGION 1..7: note = DQN0385L0605 L_CDR2
YASTKAE

SEQ ID NO: 152 - protein, 8 aa, synthetic construct
  REGION 1..8: note = DQN0385L0605 L_CDR3
HYGISKVS

SEQ ID NO: 153 - protein, 6 aa, synthetic construct
  REGION 1..6: note = DQN0385H1255 H_CDR1
EWYFMS

SEQ ID NO: 154 - protein, 17 aa, synthetic construct
  REGION 1..17: note = DQN0385H1255 H_CDR2
SIDTGSGSIDYAGWVEE

SEQ ID NO: 155 - protein, 8 aa, synthetic construct
  REGION 1..8: note = DQN0385H1255 H_CDR3
DIGIDYNF

SEQ ID NO: 156 - protein, 6 aa, synthetic construct
  REGION 1..6: note = DQN0385H1521 H_CDR1
SWYFMS

SEQ ID NO: 157 - protein, 17 aa, synthetic construct
  REGION 1..17: note = DQN0385H1521 H_CDR2
SIDTGSGSIDYAEWVEG

SEQ ID NO: 158 - protein, 8 aa, synthetic construct
  REGION 1..8: note = DQN0385H1521 H_CDR3
DIGIDYNF

SEQ ID NO: 159 - protein, 6 aa, synthetic construct
  REGION 1..6: note = DQN0385H1353 H_CDR1
EWYFMS

SEQ ID NO: 160 - protein, 17 aa, synthetic construct
  REGION 1..17: note = DQN0385H1353 H_CDR2
SIDTGSGSIDYAEWVEG

SEQ ID NO: 161 - protein, 8 aa, synthetic construct
  REGION 1..8: note = DQN0385H1353 H_CDR3
DIGIDYNF

SEQ ID NO: 162 - protein, 328 aa, synthetic construct
  REGION 1..328: note = SG1399.A5
ASTKGPSVFPLAPSSKSTSGGTAALGCLVKDYFPEPVTVSWNSGALTSGVHTFPAVLKSSGLYSLSSVVTVPSSSLGTQTYICNVNHKPSNTKVDKRVEPKSCDKTHTCPPCPAPELRRGPSVFLFPPKPKDTLMISRTPEVTCVVVDVSHEDPEVKFNWYVDGVEVHNAKTKPREEQYNSTYRVVSVLTVLHQDWLNGKEYKCKVSNKALPAPIEKTISKAKGQPREPQVYTLPPSREEMTKNQVSLTCLVKGFYPSDIAVEWESNGQPENNYKTTPPVLDSDGSFFLYSKLTVDKSRWQEGNVFSCSVLHEALHAHYTREELSLSP

SEQ ID NO: 163 - protein, 328 aa, synthetic construct
  REGION 1..328: note = SG1398.A5
ASTKGPSVFPLAPSSKSTSGGTAALGCLVEDYFPEPVTVSWNSGALTSGVHTFPAVLESSGLYSLSSVVTVPSSSLGTKTYICNVNHKPSNTKVDKRVEPKSCDKTHTCPPCPAPELRRGPSVFLFPPKPKDTLMISRTPEVTCVVVDVSHEDPEVKFNWYVDGVEVHNAKTKPREEQYNSTYRVVSVLTVLHQDWLNGKEYKCKVSNKALPAPIEKTISKAKGQPREPQVYTLPPSRKEMTKNQVSLTCLVKGFYPSDIAVEWESNGQPENNYKTTPPVLDSDGSFFLYSKLTVDKSRWQQGNVFSCSVLHEALHAHYTRKELSLSP

SEQ ID NO: 164 - protein, 6 aa, synthetic construct
  REGION 1..6: note = DQN0344H1013 H_CDR1
SAYWMV

SEQ ID NO: 165 - protein, 17 aa, synthetic construct
  REGION 1..17: note = DQN0344H1013 H_CDR2
AVYGGSDTTYYAKWTEG

SEQ ID NO: 166 - protein, 13 aa, synthetic construct
  REGION 1..13: note = DQN0344H1013 H_CDR3
EPLNYYYYGELNV

SEQ ID NO: 167 - protein, 11 aa, synthetic construct
  REGION 1..11: note = DQN0344L0620 L_CDR1
QATENIYSGLA

SEQ ID NO: 168 - protein, 7 aa, synthetic construct
  REGION 1..7: note = DQN0344L0620 L_CDR2
YVSTLAY

SEQ ID NO: 169 - protein, 10 aa, synthetic construct
  REGION 1..10: note = DQN0344L0620 L_CDR3
QTYEDVSAVT

SEQ ID NO: 170 - protein, 19 aa, synthetic construct
  REGION 1..19: note = CAMPATH-1H signal sequence
MGWSCIILFLVATATGVHS

SEQ ID NO: 171 - protein, 4 aa, synthetic construct
  REGION 1..4: note = GGGG linker
GGGG

SEQ ID NO: 172 - protein, 33 aa, synthetic construct
  REGION 1..33: note = 33-mer gliadin peptide
LQLQPFPQPELPYPQPELPYPQPELPYPQPQPF

SEQ ID NO: 173 - protein, 5 aa, synthetic construct
  REGION 1..5: note = GGGGG linker
GGGGG

SEQ ID NO: 174 - protein, 8 aa, synthetic construct
  REGION 1..8: note = 3C protease cleavage linker
LEVLFQGP

SEQ ID NO: 175 - protein, 11 aa, synthetic construct
  REGION 1..11: note = gamma 2 gliadin peptide
IIQPEQPAQLP

SEQ ID NO: 176 - protein, 17 aa, synthetic construct
  REGION 1..17: note = BC Hordein peptide
EPEQPIPEQPQPYPQQP

SEQ ID NO: 177 - protein, 29 aa, synthetic construct
  REGION 1..29: note = CLIP peptide
KLPKPPKPVSKMRMATPLLMQALPMGALP

SEQ ID NO: 178 - protein, 15 aa, synthetic construct
  REGION 1..15: note = Hepatits B virus peptide
PDRVHFASPLHVAWR

SEQ ID NO: 179 - protein, 9 aa, synthetic construct
  REGION 1..9: note = Salmonella peptide
MMAWRMMRY

SEQ ID NO: 180 - protein, 16 aa, synthetic construct
  REGION 1..16: note = Thyroperoxidase peptide
YIDVWLGGLAENFLPY

SEQ ID NO: 181 - protein, 14 aa, synthetic construct
  REGION 1..14: note = Mycobacterium bovis peptide
KPLLIIAEDVEGEY

SEQ ID NO: 182 - protein, 11 aa, synthetic construct
  REGION 1..11: note = alpha 1 gliadin peptide
QPFPQPELPYP

SEQ ID NO: 183 - protein, 11 aa, synthetic construct
  REGION 1..11: note = alpha 2 gliadin peptide
FPQPELPYPQP

SEQ ID NO: 184 - protein, 11 aa, synthetic construct
  REGION 1..11: note = gamma 1 gliadin peptide
QPQQSFPEQQQ

SEQ ID NO: 185 - protein, 12 aa, synthetic construct
  REGION 1..12: note = gamma 2 gliadin peptide
GIIQPEQPAQLP

SEQ ID NO: 186 - protein, 11 aa, synthetic construct
  REGION 1..11: note = omega 1 gliadin peptide
QPFPQPEQPFP

SEQ ID NO: 187 - protein, 11 aa, synthetic construct
  REGION 1..11: note = omega 2 gliadin peptide
FPQPEQPFPWQ

SEQ ID NO: 188 - protein, 16 aa, synthetic construct
  REGION 1..16: note = BC hordein peptide
PQQPIPEQPQPYPQQP

SEQ ID NO: 189 - protein, 11 aa, synthetic construct
  REGION 1..11: note = alpha 3 gliadin peptide
PFRPEQPYPQP

SEQ ID NO: 190 - protein, 11 aa, synthetic construct
  REGION 1..11: note = alpha 1b gliadin peptide
LPYPQPELPYP

SEQ ID NO: 191 - protein, 11 aa, synthetic construct
  REGION 1..11: note = gamma 4a gliadin peptide
FSQPEQEFPQP

SEQ ID NO: 192 - protein, 11 aa, synthetic construct
  REGION 1..11: note = gamma 4b gliadin peptide
FPQPEQEFPQP

SEQ ID NO: 193 - protein, 11 aa, synthetic construct
  REGION 1..11: note = avenin 1 peptide
QPYPEQEEPFV

SEQ ID NO: 194 - protein, 11 aa, synthetic construct
  REGION 1..11: note = avenin 2 peptide
QPYPEQEQPFV

SEQ ID NO: 195 - protein, 11 aa, synthetic construct
  REGION 1..11: note = avenin 3 peptide
QPYPEQEQPIL

SEQ ID NO: 196 - protein, 14 aa, synthetic construct
  REGION 1..14: note = hordein 1 peptide
PQQPFPQPEQPFRQ

SEQ ID NO: 197 - protein, 14 aa, synthetic construct
  REGION 1..14: note = hordein 2 peptide
QEFPQPEQPFPQQP

SEQ ID NO: 198 - protein, 14 aa, synthetic construct
  REGION 1..14: note = secalin 1 peptide
PEQPFPQPEQPFPQ

SEQ ID NO: 199 - protein, 14 aa, synthetic construct
  REGION 1..14: note = secalin 2 peptide
QPFPQPEQPFPQSQ

SEQ ID NO: 200 - protein, 15 aa, synthetic construct
  REGION 1..15: note = 14mer 1 gliadin peptide
PQQQTLQPEQPAQLP

SEQ ID NO: 201 - protein, 33 aa, synthetic construct; identical to SEQ ID NO: 172
  REGION 1..33: note = 33mer gliadin peptide

SEQ ID NO: 202 - protein, 26 aa, synthetic construct
  REGION 1..26: note = 26mer gliadin peptide
FLQPEQPFPEQPEQPYPEQPEQPFPQ

SEQ ID NO: 203 - protein, 22 aa, synthetic construct
  REGION 1..22: note = P2A
GSGATNFSLLKQAGDVEENPGP

SEQ ID NO: 204 - protein, 15 aa, synthetic construct
  REGION 1..15: note = omega1/2 gliadin peptide
EQPFPQPEQPFPWQP

SEQ ID NO: 205 - protein, 16 aa, synthetic construct
  REGION 1..16: note = BC hordein peptide
EPEQPIPEQPQPYPQQ

SEQ ID NO: 206 - protein, 15 aa, synthetic construct
  REGION 1..15: note = gamma 1 gliadin peptide
PQQPQQSFPEQEQPA

SEQ ID NO: 207 - protein, 15 aa, synthetic construct
  REGION 1..15: note = gamma 2 gliadin peptide
GQGIIQPEQPAQLIR

SEQ ID NO: 208 - protein, 23 aa, synthetic construct
  REGION 1..23: note = gamma 3 gliadin peptide
EQPFPEQPEQPYPEQPEQPFPQP

SEQ ID NO: 209 - protein, 12 aa, synthetic construct
  REGION 1..12: note = gamma 4a gliadin peptide
FSQPEQEFPQPQ

SEQ ID NO: 210 - protein, 20 aa, synthetic construct
  REGION 1..20: note = gamma 4d gliadin peptide
WPQQQPFPQPEQPFCEQPQR